European Patent Application EP 4 119 570 A1, published January 18, 2023. Title: COMPOSITION FOR ANTI-DIABETES AND ANTI-OBESITY COMPRISING NOVEL COMPOUND. Applicant: ANYGEN CO., LTD. The sequence listing filed with the application follows.

SEQUENCE LISTING (19 sequences)

SEQ ID NO: 1 - protein, 4 aa, Artificial Sequence
  HKFY protein
HKFY

SEQ ID NO: 2 - protein, 6 aa, Artificial Sequence
  Gly-Ser-His(trt)-Lys(caprylic)-Phe-Tyr
GSHKFY

SEQ ID NO: 3 - protein, 11 aa, Artificial Sequence
  His(trt)-Lys(caprylic)-Phe-Tyr-Ser-Asp-Gln-Gln-Ala-Arg-Phe
HKFYSDQQARF

SEQ ID NO: 4 - protein, 11 aa, Artificial Sequence
  His(trt)-Lys(caprylic)-Phe-Tyr-Ser-Gln-Asn-Gly-Ala-Arg-Phe
HKFYSQNGARF

SEQ ID NO: 5 - protein, 11 aa, Artificial Sequence
  His(trt)-Lys(caprylic)-Phe-Tyr-Ser-His-Gln-Gln-Ala-Arg-Phe
HKFYSHQQARF

SEQ ID NO: 6 - protein, 10 aa, Artificial Sequence
  His(trt)-Lys(caprylic)-Phe-Tyr-Gln-Asn-Gly-Ala-Arg-Phe
HKFYQNGARF

SEQ ID NO: 7 - protein, 10 aa, Artificial Sequence
  His(trt)-Lys(caprylic)-Phe-Tyr-His-Gln-Gln-Ala-Arg-Phe
HKFYHQQARF

SEQ ID NO: 8 - protein, 10 aa, Artificial Sequence
  His(trt)-Lys(caprylic)-Phe-Tyr-Gln-Asn-Gln-Ala-Arg-Phe
HKFYQNQARF

SEQ ID NO: 9 - protein, 5 aa, Artificial Sequence
  His(trt)-Lys(caprylic)-Phe-Tyr-Trp
HKFYW

SEQ ID NO: 10 - protein, 4 aa, Artificial Sequence
  Biotin-His(trt)-Lys(caprylic)-Bip-Tyr
HKAY

SEQ ID NO: 11 - protein, 4 aa, Artificial Sequence
  His(trt)-Lys(caprylic)-Phe-Trp
HKFW

SEQ ID NO: 12 - protein, 4 aa, Artificial Sequence
  His(trt)-Lys(caprylic)-Tyr-Phe
HKYF

SEQ ID NO: 13 - protein, 4 aa, Artificial Sequence
  His(trt)-Lys(caprylic)-Tyr-Tyr
HKYY

SEQ ID NO: 14 - protein, 4 aa, Artificial Sequence
  His(trt)-Lys(caprylic)-Phe-Ser
HKFS

SEQ ID NO: 15 - protein, 4 aa, Artificial Sequence
  His(trt)-Lys(caprylic)-Leu-Tyr
HKLY

SEQ ID NO: 16 - protein, 9 aa, Artificial Sequence
  His(trt)-Phe-Tyr-Asp-Gln-Gln-Ala-Arg-Phe
HFYDQQARF

SEQ ID NO: 17 - protein, 6 aa, Artificial Sequence
  His(trt)-Gly-Ser-Lys(caprylic)-Phe-Tyr
HGSKFY

SEQ ID NO: 18 - protein, 4 aa, Artificial Sequence
  Lys(caprylic)-His(trt)-Phe-Tyr
KHFY

SEQ ID NO: 19 - protein, 10 aa, Artificial Sequence
  His(trt)-Lys(caproic)-Phe-Tyr-Asp-Gln-Gln-Ala-Arg-Phe
HKFYDQQARF